European Patent Application EP 4 339 209 A1, published March 20, 2024. Title: Anti-GITR antibodies and uses thereof. Applicant: MediMabBio Inc. The sequence listing filed with the application follows.

SEQUENCE LISTING (36 sequences)

SEQ ID NO: 1 - protein, 5 aa, Artificial Sequence
  Synthetic_CDR-H1, wherein X is E, N, or D
GYWIX

SEQ ID NO: 2 - protein, 17 aa, Artificial Sequence
  Synthetic_CDR-H2
EILPGSGATYYSENFKG

SEQ ID NO: 3 - protein, 9 aa, Artificial Sequence
  Synthetic_CDR-H3
KGGYYAMDY

SEQ ID NO: 4 - protein, 12 aa, Artificial Sequence
  Synthetic_CDR-L1
TASSSVSSSYFH

SEQ ID NO: 5 - protein, 7 aa, Artificial Sequence
  Synthetic_CDR-L2, wherein X is A, Q, or E
STSNLXS

SEQ ID NO: 6 - protein, 9 aa, Artificial Sequence
  Synthetic_CDR-L3
HLYHRSPRT

SEQ ID NO: 7 - protein, 5 aa, Artificial Sequence
  Synthetic_CDR-H1
GYWIE

SEQ ID NO: 8 - protein, 5 aa, Artificial Sequence
  Synthetic_CDR-H1
GYWIN

SEQ ID NO: 9 - protein, 5 aa, Artificial Sequence
  Synthetic_CDR-H1
GYWID

SEQ ID NO: 10 - protein, 7 aa, Artificial Sequence
  Synthetic_CDR-L2
STSNLAS

SEQ ID NO: 11 - protein, 7 aa, Artificial Sequence
  Synthetic_CDR-L2
STSNLQS

SEQ ID NO: 12 - protein, 7 aa, Artificial Sequence
  Synthetic_CDR-L2
STSNLES

SEQ ID NO: 13 - protein, 118 aa, Artificial Sequence
  Synthetic_Heavy chain variable region
QVQLQQSGAELMKPGASVKLSCKTTGYRFTGYWIEWVKQRPGHGLEWIGEILPGSGATYYSENFKGKATFTADTSSNTAYMQVSSLTTGDSAIYYCARKGGYYAMDYWGQGTSVTVSS

SEQ ID NO: 14 - protein, 118 aa, Artificial Sequence
  Synthetic_Heavy chain variable region
QVQLVQSGAELKKPGASVKLSCKTTGYRFTGYWIEWVRQPPGKGLEWIGEILPGSGATYYSENFKGKATITADTSTNTAYMEVSSLRSGDSAIYYCARKGGYYAMDYWGQGTSVTVSS

SEQ ID NO: 15 - protein, 118 aa, Artificial Sequence
  Synthetic_Heavy chain variable region
QVQLVQSGAEVKKPGASVKLSCKTTGYRFTGYWIEWVRQPPGKGLEWIGEILPGSGATYYSENFKGKATITADTSTNTAYMEVSSLRSEDTAIYYCARKGGYYAMDYWGQGTLVTVSS

SEQ ID NO: 16 - protein, 118 aa, Artificial Sequence
  Synthetic_Heavy chain variable region
QVQLVQSGAEVKKPGASVKVSCKTTGYRFTGYWIEWVRQPPGKGLEWIGEILPGSGATYYSENFKGKVTITADTSTDTAYMELSSLRSEDTAIYYCARKGGYYAMDYWGQGTLVTVSS

SEQ ID NO: 17 - protein, 118 aa, Artificial Sequence
  Synthetic_Heavy chain variable region
QVQLVQSGAEVKKPGASVKVSCKTTGYRFTGYWINWVRQPPGKGLEWIGEILPGSGATYYSENFKGKVTITADTSTDTAYMELSSLRSEDTAIYYCARKGGYYAMDYWGQGTLVTVSS

SEQ ID NO: 18 - protein, 118 aa, Artificial Sequence
  Synthetic_Heavy chain variable region
QVQLVQSGAEVKKPGASVKVSCKTTGYRFTGYWIDWVRQPPGKGLEWIGEILPGSGATYYSENFKGKVTITADTSTDTAYMELSSLRSEDTAIYYCARKGGYYAMDYWGQGTLVTVSS

SEQ ID NO: 19 - protein, 108 aa, Artificial Sequence
  Synthetic_Light chain variable region
QIVLTQSPAIMSASLGERVTMTCTASSSVSSSYFHWYQQKPGSSPKLWIYSTSNLASGVPARFSGSGSGTSYSLTVSSLEAEDAATYYCHLYHRSPRTFGGGTTLDIK

SEQ ID NO: 20 - protein, 108 aa, Artificial Sequence
  Synthetic_Light chain variable region
QIVLTQSPAIMSASLGERVTMSCTASSSVSSSYFHWYQQKPGSAPKLWIYSTSNLASGVPDRFSGSGSGTDYTLTVSSLQAEDVATYYCHLYHRSPRTFGGGTTVDIK

SEQ ID NO: 21 - protein, 108 aa, Artificial Sequence
  Synthetic_Light chain variable region
QIVLTQSPATLSLSPGERATMSCTASSSVSSSYFHWYQQKPGSAPKLWIYSTSNLASGVPDRFSGSGSGTDYTLTISSLQAEDVATYYCHLYHRSPRTFGGGTKVEIK

SEQ ID NO: 22 - protein, 108 aa, Artificial Sequence
  Synthetic_Light chain variable region
EIVLTQSPATLSLSPGERATLSCTASSSVSSSYFHWYQQKPGSAPKLWIYSTSNLASGVPDRFSGSGSGTDYTLTISSLQAEDVATYYCHLYHRSPRTFGGGTKVEIK

SEQ ID NO: 23 - protein, 108 aa, Artificial Sequence
  Synthetic_Light chain variable region
EIVLTQSPATLSLSPGERATLSCTASSSVSSSYFHWYQQKPGKAPKLWIYSTSNLQSGVPDRFSGSGSGTDYTLTISSLQAEDVATYYCHLYHRSPRTFGGGTKVEIK

SEQ ID NO: 24 - protein, 108 aa, Artificial Sequence
  Synthetic_Light chain variable region
EIVLTQSPATLSLSPGERATLSCTASSSVSSSYFHWYQQKPGKAPKLWIYSTSNLESGVPDRFSGSGSGTDYTLTISSLQAEDVATYYCHLYHRSPRTFGGGTKVEIK

SEQ ID NO: 25 - protein, 330 aa, Artificial Sequence
  Synthetic_Heavy chain constant region
ASTKGPSVFPLAPSSKSTSGGTAALGCLVKDYFPEPVTVSWNSGALTSGVHTFPAVLQSSGLYSLSSVVTVPSSSLGTQTYICNVNHKPSNTKVDKRVEPKSCDKTHTCPPCPAPELLGGPSVFLFPPKPKDTLMISRTPEVTCVVVDVSHEDPEVKFNWYVDGVEVHNAKTKPREEQYNSTYRVVSVLTVLHQDWLNGKEYKCKVSNKALPAPIEKTISKAKGQPREPQVYTLPPSREEMTKNQVSLTCLVKGFYPSDIAVEWESNGQPENNYKTTPPVLDSDGSFFLYSKLTVDKSRWQQGNVFSCSVMHEALHNHYTQKSLSLSPGK

SEQ ID NO: 26 - protein, 107 aa, Artificial Sequence [sequence omitted]

SEQ ID NO: 27 - protein, 448 aa, Artificial Sequence
  Synthetic_51B chimeric N298A_VH (Heavy chain)
QVQLQQSGAELMKPGASVKLSCKTTGYRFTGYWIEWVKQRPGHGLEWIGEILPGSGATYYSENFKGKATFTADTSSNTAYMQVSSLTTGDSAIYYCARKGGYYAMDYWGQGTSVTVSSASTKGPSVFPLAPSSKSTSGGTAALGCLVKDYFPEPVTVSWNSGALTSGVHTFPAVLQSSGLYSLSSVVTVPSSSLGTQTYICNVNHKPSNTKVDKRVEPKSCDKTHTCPPCPAPELLGGPSVFLFPPKPKDTLMISRTPEVTCVVVDVSHEDPEVKFNWYVDGVEVHNAKTKPREEQYASTYRVVSVLTVLHQDWLNGKEYKCKVSNKALPAPIEKTISKAKGQPREPQVYTLPPSREEMTKNQVSLTCLVKGFYPSDIAVEWESNGQPENNYKTTPPVLDSDGSFFLYSKLTVDKSRWQQGNVFSCSVMHEALHNHYTQKSLSLSPGK

SEQ ID NO: 28 - protein, 215 aa, Artificial Sequence
  Synthetic_51B chimeric N298A_VL (Light chain)
QIVLTQSPAIMSASLGERVTMTCTASSSVSSSYFHWYQQKPGSSPKLWIYSTSNLASGVPARFSGSGSGTSYSLTVSSLEAEDAATYYCHLYHRSPRTFGGGTTLDIKRTVAAPSVFIFPPSDEQLKSGTASVVCLLNNFYPREAKVQWKVDNALQSGNSQESVTEQDSKDSTYSLSSTLTLSKADYEKHKVYACEVTHQGLSSPVTKSFNRGEC

SEQ ID NO: 29 - protein, 137 aa, Artificial Sequence
  Synthetic_51B heavy chain variable region comprising signal sequence, wherein the amino acid sequecen of 1-19 is signal sequence
MEWTWVFLFLLSVTAGVHSQVQLQQSGAELMKPGASVKLSCKTTGYRFTGYWIEWVKQRPGHGLEWIGEILPGSGATYYSENFKGKATFTADTSSNTAYMQVSSLTTGDSAIYYCARKGGYYAMDYWGQGTSVTVSS

SEQ ID NO: 30 - DNA, 411 bp, Artificial Sequence
  Synthetic_DNA encoding 51B heavy chain variable region comprising signal sequence
atggaatggacctgggtctttctcttcctcctgtcagtaactgcaggtgtccactcccaggttcagctgcagcagtctggagctgagctgatgaagcctggggcctcagtgaagctttcctgcaagactactggctacagattcactggctactggatagagtgggtaaaacaaaggcctggacatggccttgagtggatcggagagattttacctggaagtggtgctacttactacagtgagaacttcaagggcaaggccacattcactgcagatacatcctccaacacagcctacatgcaagtcagcagcctgacaactggggactctgccatctattattgtgcaagaaagggggggtactatgctatggactactggggtcaaggaacctcagtcaccgtctcctca

SEQ ID NO: 31 - protein, 130 aa, Artificial Sequence
  Synthetic_51B light chain variable region comprising signal sequence, wherein the amino acid sequecen of 1-22 is signal sequence
MDFQVQIFSFLLISASVIMSRGQIVLTQSPAIMSASLGERVTMTCTASSSVSSSYFHWYQQKPGSSPKLWIYSTSNLASGVPARFSGSGSGTSYSLTVSSLEAEDAATYYCHLYHRSPRTFGGGTTLDIK

SEQ ID NO: 32 - DNA, 390 bp, Artificial Sequence
  Synthetic_DNA encoding 51B light chain variable region comprising signal sequence
atggattttcaggtgcagattttcagcttcctgctaatcagtgcctcagtcataatgtccagaggacaaattgttctcacccagtctccagcaatcatgtctgcatctctaggggaacgggtcaccatgacctgcactgccagctcaagtgtaagttccagttattttcactggtaccagcagaagccaggatcctcacccaaactctggatttatagcacttccaacctggcttctggagtcccagctcgcttcagtggcagtgggtctgggacctcttactctctcacagtcagcagtttggaggctgaggatgctgccacttattactgccacctgtatcatcgttccccacggacgttcggtggaggcaccacgctggatatcaaa

SEQ ID NO: 33 - protein, 241 aa, Artificial Sequence
  Synthetic_human GITR, wherein the aminno acid sequence of amino acids 1-25 is signal sequence
MAQHGAMGAFRALCGLALLCALSLGQRPTGGPGCGPGRLLLGTGTDARCCRVHTTRCCRDYPGEECCSEWDCMCVQPEFHCGDPCCTTCRHHPCPPGQGVQSQGKFSFGFQCIDCASGTFSGGHEGHCKPWTDCTQFGFLTVFPGNKTHNAVCVPGSPPAEPLGWLTVVLLAVAACVLLLTSAQLGLHIWQLRSQCMWPRETQLLLEVPPSTEDARSCQFPEEERGERSAEEKGRLGDLWV

SEQ ID NO: 34 - protein, 5 aa, Artificial Sequence
  Synthetic_Epitope region on human GITR
SGTFS

SEQ ID NO: 35 - protein, 10 aa, Artificial Sequence
  Synthetic_Epitope region on human GITR
TDCTQFGFLT

SEQ ID NO: 36 - protein, 11 aa, Artificial Sequence
  Synthetic_Epitope region on human GITR
KTHNAVCVPGS